European Patent Application EP 4 582 544 A1, published July 9, 2025. Title: 光応答改変型オプシン類. Applicant: 国立大学法人京都大学. Application JP. The sequence listing filed with the application follows.

SEQUENCE LISTING (68 sequences)

SEQ ID NO: 1 - protein, 348 aa, Homo sapiens [sequence omitted]

SEQ ID NO: 2 - protein, 348 aa, Mus musculus
MNGTEGPNFYVPFSNVTGVVRSPFEQPQYYLAEPWQFSMLAAYMFLLIVLGFPINFLTLYVTVQHKKLRTPLNYILLNLAVADLFMVFGGFTTTLYTSLHGYFVFGPTGCNLEGFFATLGGEIALWSLVVLAIERYVVVCKPMSNFRFGENHAIMGVVFTWIMALACAAPPLVGWSRYIPEGMQCSCGIDYYTLKPEVNNESFVIYMFVVHFTIPMIVIFFCYGQLVFTVKEAAAQQQESATTQKAEKEVTRMVIIMVIFFLICWLPYASVAFYIFTHQGSNFGPIFMTLPAFFAKSSSIYNPVIYIMLNKQFRNCMLTTLCCGKNPLGDDDASATASKTETSQVAPA

SEQ ID NO: 3 - protein, 348 aa, Canis familiaris
MNGTEGPNFYVPFSNKTGVVRSPFEYPQYYLAEPWQFSMLAAYMFLLIVLGFPINFLTLYVTVQHKKLRTPLNYILLNLAVADLFMVFGGFTTTLYTSLHGYFVFGPTGCNVEGFFATLGGEIALWSLVVLAIERYVVVCKPMSNFRFGENHAIMGVAFTWVMALACAAPPLAGWSRYIPEGMQCSCGIDYYTLKPEINNESFVIYMFVVHFAIPMIVIFFCYGQLVFTVKEAAAQQQESATTQKAEKEVTRMVIIMVIAFLICWVPYASVAFYIFTHQGSDFGPIFMTLPAFFAKSSSIYNPVIYIMMNKQFRNCMITTLCCGKNPLGDDEASASASKTETSQVAPA

SEQ ID NO: 4 - protein, 351 aa, Gallus gallus
MNGTEGQDFYVPMSNKTGVVRSPFEYPQYYLAEPWKFSALAAYMFMLILLGFPVNFLTLYVTIQHKKLRTPLNYILLNLAVADLFMVFGGFTTTMYTSMNGYFVFGVTGCYIEGFFATLGGEIALWSLVVLAVERYVVVCKPMSNFRFGENHAIMGVAFSWIMAMACAAPPLFGWSRYIPEGMQCSCGIDYYTLKPEINNESFVIYMFVVHFMIPLAVIFFCYGNLVCTVKEAAAQQQESATTQKAEKEVTRMVIIMVIAFLICWVPYASVAFYIFTNQGSDFGPIFMTIPAFFAKSSAIYNPVIYIVMNKQFRNCMITTLCCGKNPLGDEDTSAGKTETSSVSTSQVSPA

SEQ ID NO: 5 - protein, 354 aa, Oryzias latipes
MNGTEGPYFYVPMVNTTGIVRSPYEYPQYYLVNPAAYAALGAYMFFLILVGFPINFLTLYVTLEHKKLRTPLNYILLNLAVADLFMVFGGFTTTMYTSMHGYFVLGRLGCNLEGFFATLGGEIGLWSLVVLAIERWVVVCKPISNFRFGENHAIMGLVFTWIMAASCAVPPLVGWSRYIPEGMQCSCGVDYYTRAEGFNNESFVVYMFVCHFLIPLIVVFFCYGRLLCAVKEAAAAQQESETTQRAEREVTRMVVIMVIGFLVCWLPYASVAWYIFTNQGSEFGPLFMTIPAFFAKSSSIYNPAIYICMNKQFRNCMITTLCCGKNPFEEEEGASTTASKTEASSVSSSSVSPA

SEQ ID NO: 6 - protein, 348 aa, Homo sapiens
MRKMSEEEFYLFKNISSVGPWDGPQYHIAPVWAFYLQAAFMGTVFLIGFPLNAMVLVATLRYKKLRQPLNYILVNVSFGGFLLCIFSVFPVFVASCNGYFVFGRHVCALEGFLGTVAGLVTGWSLAFLAFERYIVICKPFGNFRFSSKHALTVVLATWTIGIGVSIPPFFGWSRFIPEGLQCSCGPDWYTVGTKYRSESYTWFLFIFCFIVPLSLICFSYTQLLRALKAVAAQQQESATTQKAEREVSRMVVVMVGSFCVCYVPYAAFAMYMVNNRNHGLDLRLVTIPSFFSKSACIYNPIIYCFMNKQFQACIMKMVCGKAMTDESDTCSSQKTEVSTVSSTQVGPN

SEQ ID NO: 7 - protein, 364 aa, Homo sapiens
MAQQWSLQRLAGRHPQDSYEDSTQSSIFTYTNSNSTRGPFEGPNYHIAPRWVYHLTSVWMIFVVTASVFTNGLVLAATMKFKKLRHPLNWILVNLAVADLAETVIASTISIVNQVSGYFVLGHPMCVLEGYTVSLCGITGLWSLAIISWERWMVVCKPFGNVRFDAKLAIVGIAFSWIWAAVWTAPPIFGWSRYWPHGLKTSCGPDVFSGSSYPGVQSYMIVLMVTCCIIPLAIIMLCYLQVWLAIRAVAKQQKESESTQKAEKEVTRMVVVMIFAYCVCWGPYTFFACFAAANPGYAFHPLMAALPAYFAKSATIYNPVIYVFMNRQFRNCILQLFGKKVDDGSELSSASKTEVSSVSSVSPA

SEQ ID NO: 8 - protein, 364 aa, Homo sapiens
MAQQWSLQRLAGRHPQDSYEDSTQSSIFTYTNSNSTRGPFEGPNYHIAPRWVYHLTSVWMIFVVIASVFTNGLVLAATMKFKKLRHPLNWILVNLAVADLAETVIASTISVVNQVYGYFVLGHPMCVLEGYTVSLCGITGLWSLAIISWERWMVVCKPFGNVRFDAKLAIVGIAFSWIWAAVWTAPPIFGWSRYWPHGLKTSCGPDVFSGSSYPGVQSYMIVLMVTCCITPLSIIVLCYLQVWLAIRAVAKQQKESESTQKAEKEVTRMVVVMVLAFCFCWGPYAFFACFAAANPGYPFHPLMAALPAFFAKSATIYNPVIYVFMNRQFRNCILQLFGKKVDDGSELSSASKTEVSSVSSVSPA

SEQ ID NO: 9 - protein, 346 aa, Mus musculus
MSGEDDFYLFQNISSVGPWDGPQYHLAPVWAFRLQAAFMGFVFFVGTPLNAIVLVATLHYKKLRQPLNYILVNVSLGGFLFCIFSVFTVFIASCHGYFLFGRHVCALEAFLGSVAGLVTGWSLAFLAFERYVVICKPFGSIRFNSKHALMVVLATWIIGIGVSIPPFFGWSRFIPEGLQCSCGPDWYTVGTKYRSEYYTWFLFIFCFIIPLSLICFSYSQLLRTLRAVAAQQQESATTQKAEREVSHMVVVMVGSFCLCYVPYAALAMYMVNNRNHGLDLRLVTIPAFFSKSSCVYNPIIYCFMNKQFRACILEMVCRKPMADESDVSGSQKTEVSTVSSSKVGPH

SEQ ID NO: 10 - protein, 359 aa, Mus musculus
MAQRLTGEQTLDHYEDSTHASIFTYTNSNSTKGPFEGPNYHIAPRWVYHLTSTWMILVVVASVFTNGLVLAATMRFKKLRHPLNWILVNLAVADLAETIIASTISVVNQIYGYFVLGHPLCVIEGYIVSLCGITGLWSLAIISWERWLVVCKPFGNVRFDAKLATVGIVFSWVWAAIWTAPPIFGWSRYWPYGLKTSCGPDVFSGTSYPGVQSYMMVLMVTCCIFPLSIIVLCYLQVWLAIRAVAKQQKESESTQKAEKEVTRMVVVMVFAYCLCWGPYTFFACFATAHPGYAFHPLVASLPSYFAKSATIYNPIIYVFMNRQFRNCILHLFGKKVDDSSELSSTSKTEVSSVSSVSPA

SEQ ID NO: 11 - protein, 355 aa, Gallus gallus
MNGTEGINFYVPMSNKTGVVRSPFEYPQYYLAEPWKYRLVCCYIFFLISTGLPINLLTLLVTFKHKKLRQPLNYILVNLAVADLFMACFGFTVTFYTAWNGYFVFGPVGCAVEGFFATLGGQVALWSLVVLAIERYIVVCKPMGNFRFSATHAMMGIAFTWVMAFSCAAPPLFGWSRYMPEGMQCSCGPDYYTHNPDYHNESYVLYMFVIHFIIPVVVIFFSYGRLICKVREAAAQQQESATTQKAEKEVTRMVILMVLGFMLAWTPYAVVAFWIFTNKGADFTATLMAVPAFFSKSSSLYNPIIYVLMNKQFRNCMITTICCGKNPFGDEDVSSTVSQSKTEVSSVSSSQVSPA

SEQ ID NO: 12 - protein, 361 aa, Gallus gallus
MHPPRPTTDLPEDFYIPMALDAPNITALSPFLVPQTHLGSPGLFRAMAAFMFLLIALGVPINTLTIFCTARFRKLRSHLNYILVNLALANLLVILVGSTTACYSFSQMYFALGPTACKIEGFAATLGGMVSLWSLAVVAFERFLVICKPLGNFTFRGSHAVLGCVATWVLGFVASAPPLFGWSRYIPEGLQCSCGPDWYTTDNKWHNESYVLFLFTFCFGVPLAIIVFSYGRLLITLRAVARQQEQSATTQKADREVTKMVVVMVLGFLVCWAPYTAFALWVVTHRGRSFEVGLASIPSVFSKSSTVYNPVIYVLMNKQFRSCMLKLLFCGRSPFGDDEDVSGSSQATQVSSVSSSHVAPA

SEQ ID NO: 13 - protein, 347 aa, Gallus gallus
MSSDDDFYLFTNGSVPGPWDGPQYHIAPPWAFYLQTAFMGIVFAVGTPLNAVVLWVTVRYKRLRQPLNYILVNISASGFVSCVLSVFVVFVASARGYFVFGKRVCELEAFVGTHGGLVTGWSLAFLAFERYIVICKPFGNFRFSSRHALLVVVATWLIGVGVGLPPFFGWSRYMPEGLQCSCGPDWYTVGTKYRSEYYTWFLFIFCFIVPLSLIIFSYSQLLSALRAVAAQQQESATTQKAEREVSRMVVVMVGSFCLCYVPYAALAMYMVNNRDHGLDLRLVTIPAFFSKSACVYNPIIYCFMNKQFRACIMETVCGKPLTDDSDASTSAQRTEVSSVSSSQVGPT

SEQ ID NO: 14 - protein, 362 aa, Gallus gallus
MAAWEAAFAARRRHEEEDTTRDSVFTYTNSNNTRGPFEGPNYHIAPRWVYNLTSLWMIFVVAASVFTNGLVLVATWKFKKLRHPLNWILVNLAVADLGETVIASTISVINQISGYFILGHPMCVVEGYTVSACGITALWSLAIISWERWFVVCKPFGNIKFDGKLAVAGILFSWLWSCAWTAPPIFGWSRYWPHGLKTSCGPDVFSGSSDPGVQSYMVVLMVTCCFFPLAIIILCYLQVSLAIRAVAAQQKESESTQKAEKEVSRMVVVMIVAYCFCWGPYTFFACFAAANPGYAFHPLAAALPAYFAKSATIYNPIIYVFMNRQFRNCILQLFGKKVDDGSEVSTSRTEVSSVSNSSVSPA

SEQ ID NO: 15 - protein, 351 aa, Gallus gallus
MSSNSSQAPPNGTPGPFDGPQWPYQAPQSTYVGVAVLMGTVVACASVVNGLVIVVSICYKKLRSPLNYILVNLAVADLLVTLCGSSVSLSNNINGFFVFGRRMCELEGFMVSLTGIVGLWSLAILALERYVVVCRPLGDFQFQRRHAVSGCAFTWGWALLWSTPPLLGWSSYVPEGLRTSCGPNWYTGGSNNNSYILSLFVTCFVLPLSLILFSYTNLLLTLRAAAAQQKEADTTQRAEREVTRMVIVMVMAFLLCWLPYSTFALVVATHKGIIIQPVLASLPSYFSKTATVYNPIIYVFMNKQFQSCLLEMLCCGYQPQRTGKASPGTPGPHADVTAAGLRNKVMPAHPV

SEQ ID NO: 16 - protein, 402 aa, Homo sapiens
MYSGNRSGGHGYWDGGGAAGAEGPAPAGTLSPAPLFSPGTYERLALLLGSIGLLGVGNNLLVLVLYYKFQRLRTPTHLLLVNISLSDLLVSLFGVTFTFVSCLRNGWVWDTVGCVWDGFSGSLFGIVSIATLTVLAYERYIRVVHARVINFSWAWRAITYIWLYSLAWAGAPLLGWNRYILDVHGLGCTVDWKSKDANDSSFVLFLFLGCLVVPLGVIAHCYGHILYSIRMLRCVEDLQTIQVIKILKYEKKLAKMCFLMIFTFLVCWMPYIVICFLVVNGHGHLVTPTISIVSYLFAKSNTVYNPVIYVFMIRKFRRSLLQLLCLRLLRCQRPAKDLPAAGSEMQIRPIVMSQKDGDRPKKKVTFNSSSIIFIITSDESLSVDDSDKTNGSKVDVIQVRPL

SEQ ID NO: 17 - protein, 478 aa, Homo sapiens
MNPPSGPRVLPSPTQEPSCMATPAPPSWWDSSQSSISSLGRLPSISPTAPGTWAAAWVPLPTVDVPDHAHYTLGTVILLVGLTGMLGNLTVIYTFCRSRSLRTPANMFIINLAVSDFLMSFTQAPVFFTSSLYKQWLFGETGCEFYAFCGALFGISSMITLTAIALDRYLVITRPLATFGVASKRRAAFVLLGVWLYALAWSLPPFFGWSAYVPEGLLTSCSWDYMSFTPAVRAYTMLLCCFVFFLPLLIIIYCYIFIFRAIRETGRALQTFGACKGNGESLWQRQRLQSECKMAKIMLLVILLFVLSWAPYSAVALVAFAGYAHVLTPYMSSVPAVIAKASAIHNPIIYAITHPKYRVAIAQHLPCLGVLLGVSRRHSRPYPSYRSTHRSTLTSHTSNLSWISIRRRQESLGSESEVGWTHMEAAAVWGAAQQANGRSLYGQGLEDLEAKAPPRPQGHEAETPGKTKGLIPSQDPRM

SEQ ID NO: 18 - protein, 354 aa, Homo sapiens
MALNHTALPQDERLPHYLRDGDPFASKLSWEADLVAGFYLTIIGILSTFGNGYVLYMSSRRKKKLRPAEIMTINLAVCDLGISVVGKPFTIISCFCHRWVFGWIGCRWYGWAGFFFGCGSLITMTAVSLDRYLKICYLSYGVWLKRKHAYICLAAIWAYASFWTTMPLVGLGDYVPEPFGTSCTLDWWLAQASVGGQVFILNILFFCLLLPTAVIVFSYVKIIAKVKSSSKEVAHFDSRIHSSHVLEMKLTKVAMLICAGFLIAWIPYAVVSVWSAFGRPDSIPIQLSVVPTLLAKSAAMYNPIIYQVIDYKFACCQTGGLKATKKKSLEGFRLHTVTTVRKSSAVLEIHEEWE

SEQ ID NO: 19 - protein, 291 aa, Homo sapiens
MAETSALPTGFGELEVLAVGMVLLVEALSGLSLNTLTIFSFCKTPELRTPCHLLVLSLALADSGISLNALVAATSSLLRRWPYGSDGCQAHGFQGFVTALASICSSAAIAWGRYHHYCTRSQLAWNSAVSLVLFVWLSSAFWAALPLLGWGHYDYEPLGTCCTLDYSKGDRNFTSFLFTMSFFNFAMPLFITITSYSLMEQKLGKSGHLQVNTTLPARTLLLGWGPYAILYLYAVIADVTSISPKLQMVPALIAKMVPTINAINYALGNEMVCRGIWQCLSPQKREKDRTK

SEQ ID NO: 20 - protein, 337 aa, Homo sapiens
MLRNNLGNSSDSKNEDGSVFSQTEHNIVATYLIMAGMISIISNIIVLGIFIKYKELRTPTNAIIINLAVTDIGVSSIGYPMSAASDLYGSWKFGYAGCQVYAGLNIFFGMASIGLLTVVAVDRYLTICLPDVGRRMTTNTYIGLILGAWINGLFWALMPIIGWASYAPDPTGATCTINWRKNDRSFVSYTMTVIAINFIVPLTVMFYCYYHVTLSIKHHTTSDCTESLNRDWSDQIDVTKMSVIMICMFLVAWSPYSIVCLWASFGDPKKIPPPMAIIAPLFAKSSTFYNPCIYVVANKKFRRAMLAMFKCQTHQTMPVTSILPMDVSQNPLASGRI

SEQ ID NO: 21 - protein, 400 aa, Mus musculus
MYSGNRSGDQGYWEDGAGAEGAAPAGTRSPAPLFSPTAYERLALLLGCLALLGVGGNLLVLLLYSKFPRLRTPTHLFLVNLSLGDLLVSLFGVTFTFASCLRNGWVWDAVGCAWDGFSGSLFGFVSITTLTVLAYERYIRVVHARVINFSWAWRAITYIWLYSLAWAGAPLLGWNRYILDIHGLGCTVDWRSKDANDSSFVLFLFLGCLVVPVGIIAHCYGHILYSVRMLRCVEDLQTIQVIKMLRYEKKVAKMCFLMAFVFLTCWMPYIVTRFLVVNGYGHLVTPTVSIVSYLFAKSSTVYNPVIYIFMNRKFRRSLLQLLCFRLLRCQRPAKNLPAAESEMHIRPIVMSQKDGDRPKKKVTFNSSSIIFIITSDESLSVEDSDRSSASKVDVIQVRPL

SEQ ID NO: 22 - protein, 521 aa, Mus musculus
MDSPSGPRVLSSLTQDPSFTTSPALQGIWNGTQNVSVRAQLLSVSPTTSAHQAAAWVPFPTVDVPDHAHYTLGTVILLVGLTGMLGNLTVIYTFCRNRGLRTPANMFIINLAVSDFLMSVTQAPVFFASSLYKKWLFGETGCEFYAFCGAVFGITSMITLTAIAMDRYLVITRPLATIGRGSKRRTALVLLGVWLYALAWSLPPFFGWSAYVPEGLLTSCSWDYMTFTPQVRAYTMLLFCFVFFLPLLIIIFCYIFIFRAIRETGRACEGCGESPLRQRRQWQRLQSEWKMAKVALIVILLFVLSWAPYSTVALVAFAGYSHILTPYMSSVPAVIAKASAIHNPIIYAITHPKYRVAIAQHLPCLGVLLGVSGQRSHPSLSYRSTHRSTLSSQSSDLSWISGRKRQESLGSESEVGWTDTETTAAWGAAQQASGQSFCSQNLEDGELKASSSPQVQRSKTPKVPGPSTCRPMKGQGARPSSLRGDQKGRLAVCTGLSECPHPHTSQFPLAFLEDDVTLRHL

SEQ ID NO: 23 - protein, 377 aa, Mus musculus
MALNHTALPQDERLPHYLRDEDPFASKLSWEADLVAGFYLTIIGILSTFGNGYVLYMSSRRKKKLRPAEIMTINLAVCDLGISVVGKPFTIISCFCHRWVFGWFGCRWYGWAGFFFGCGSLITMTAVSLDRYLKICYLSYGVWLKRKHAYICLAVIWAYASFWTTMPLVGLGDYAPEPFGTSCTLDWWLAQASGGGQVFILSILFFCLLLPTAVIVFSYAKIIAKVKSSSKEVAHFDSRIHSSHVLEVKLTKVAMLICAGFLIAWIPYAVVSVWSAFGRPDSIPIQLSVVPTLLAKSAAMYNPIIYQVIDYRFACCQAGGLRGTKKKSLEDFRLHTVTAVRKSSAVLEIHPESSSRFTSAHVMDGESHSNDGDCGKK

SEQ ID NO: 24 - protein, 291 aa, Mus musculus
MAATRALPAGLGELEVLAVGTVLLMEALSGISLNGLTIFSFCKTPDLRTPSNLLVLSLALADTGISLNALVAAVSSLLRRWPHGSEGCQVHGFQGFATALASICGSAAVAWGRYHHYCTRRQLAWDTAIPLVLFVWMSSAFWASLPLMGWGHYDYEPVGTCCTLDYSRGDRNFISFLFTMAFFNFLVPLFITHTSYRFMEQKFSRSGHLPVNTTLPGRMLLLGWGPYALLYLYAAIADVSFISPKLQMVPALIAKTMPTINAINYALHREMVCRGTWQCLSPQKSKKDRTQ

SEQ ID NO: 25 - protein, 337 aa, Mus musculus
MLSEASDFNSSGSRSEGSVFSRTEHSVIAAYLIVAGITSILSNVVVLGIFIKYKELRTPTNAVIINLAFTDIGVSSIGYPMSAASDLHGSWKFGHAGCQIYAGLNIFFGMVSIGLLTVVAMDRYLTISCPDVGRRMTTNTYLSMILGAWINGLFWALMPIIGWASYAPDPTGATCTINWRNNDTSFVSYTMMVIVVNFIVPLTVMFYCYYHVSRSLRLYAASDCTAHLHRDWADQADVTKMSVIMILMFLLAWSPYSIVCLWACFGNPKKIPPSMAIIAPLFAKSSTFYNPCIYVAAHKKFRKAMLAMFKCQPHLAVPEPSTLPMDMPQSSLAPVRI

SEQ ID NO: 26 - protein, 359 aa, Gallus gallus
MDVFRALGNESLLSNSSGPARWDPFHHPLDSIQPWHFRLVAAVMFVVTSLSLAENLAVILVTFKFKQLRQPVNYVIVNLSVADFLVSLTGGTISFLANLKGYFYMGHWACVLEGFAVTFFGIVALWSLALLAFERYIVICRPVGNMRLRGKHAAQGIAFVWTFSFIWTIPPTMGWSSYTTSKIGTTCEPNWYSGAYNDRSYIIAFFTTCFIVPLLVILVSYGKLLQKLRKVSNTQGRLRTARKPERQVTRMVVVMIIAFLICWMPYAVFSILATAYPSIELDPHLAAIPAFFSKTATVYNPIIYVFMNKQFRMCLIQMFKCSAIETAESNMNPTSERATLTQDKRDSQLSVMAVRSTIS

SEQ ID NO: 27 - protein, 395 aa, Gallus gallus
MHSGNGTGATSRPQLAAAGHEVPGERPLFSAGTYELLALLIATIGTLGVCNNLLVLVLYYKFKRLRTPTNLFLVNISLSDLLVSVCGVSLTFMSCLRSRWVWDAAGCVWDGFSNSLFGIVSIMTLTVLAYERYIRVVHAKVIDFSWSWRAITYIWLYSLAWTGAPLLGWNRYTLEIHGLGCSMDWKSKDPNDTSFVLLFFLGCLVAPVVIMAYCYGHILYAVRMLRCVEDFQTSQVIKLLKYEKKVAKMCFLMISTFLICWMPYAVVSLLVTYGYSNLVTPTVAIIPSFFAKSSTAYNPVIYIFMSRKFRQCLLQLLCFRLMRFQRIMKEPSGAGNVKPIRPIVMSQKVGDRPKKKVTFSSSSIIFIIASDDTQQIDDNSKHNGTKVNVIQVKPL

SEQ ID NO: 28 - protein, 373 aa, Gallus gallus
MNHTWTYNLSFGAPTDPVEPRAGLSRNGHTVVAVFLGFILFFGFLNNLIVLILFCKFKTLRNPVNMLLLNISISDMLVCISGTTLSFASNIHGKWIGGEHGCRWYGFVNSCFGIVSLISLAVLSYERYSTLTLCNKRSDDYRKALLAVGGSWVYSLLWTVPPLLGWSSYGIEGAGTSCSVRWSSETAESTSYIICLFIFCLVIPVMVMMYCYGRLLYAVKQVGKIHKNTARKREYHVLFMVITTVICYLVCWIPYGVIALLATFGKPGVVTPVASIIPSILAKSSTVCNPIIYILMNKQFYKCFRQLFHCQPPSSTDGEPTCHSKVTVIQLNQKTDGGKLCNNKPRPETDNKVTSLLHPEPGLEPAAKTVPPM

SEQ ID NO: 29 - protein, 543 aa, Gallus gallus
MDLNMGTQPHSVTKSEIPDHVLYTVGTCVLVIGSIGIIGNLLVLYAFYSNKKLRTPQNFFIMNLAVSDFLMSASQAPICFINSLHREWILGDIGCDLYAFCGALFGITSMMTLLAISVDRYLVITKPLRSIQWTSKKRTIQIIAAVWLYSLGWSVAPLLGWSSYVPEGLMISCTWDYVTYSPANRSYTMILCCCVFFIPLIIILHCYLFMFLAIRSTGRDVQKLGSCSRKSFLSQSMKNEWKLAKIAFVVIIVYVLSWSPYACVTLIAWAGRGNTLTPYSKSVPAVIAKASAIYNPIIYAIIHPRYRKTIHNAVPCLRFLIRISKNDLLRGSINESSFRTSLSSHQSLAGRTKNTCVSSVSTGEANWSDVELDTVEPAHEKLQPRRSHSFSSSLRQKRDLLPDSYSCSEETEEKVSLSSSYLEKVLGRSAFPSSPVALVTSSLRAASLPVGLNSSSASRGAGSDISQMKTEESHNNGGLDSIVSNTVPQIIIIPTSETNLFQEEPEEEETELFHFHDKKNNLLDLEGLSSSTEFLEAVEKFLS

SEQ ID NO: 30 - protein, 528 aa, Gallus gallus
MDLPPRAPTKMTVKDVRGAFPTVDVPDHAHYTIGTVILIVGITGTLGNFLVIYAFCRSRTLQKPANIFIINLAVSDFLMSITQSPVFFTNSLHKRWIFGEKGCELYAFCGALFGITSMITLMVIALDRYFVITKPLASVRVMSKKKALIILVGVWLYSLAWSLPPFFGWSAYVPEGLLTSCSWDYMTFTPSVRAYTMLLFCFVFFIPLIAIIYSYVFIFEAIKKANKSVQTFGCKHGNRELQKQYHRMRNEWKLAKIALIVILLYVISWSPYSVVALVAFAGYSHVLTPFMNSVPAVIAKASAIHNPIIYAITHPKYRTAIATYVPCLGFLLRVSPKESRSFSSYPSSRRTTITSQSSETSGLQKGKRRLSSISDSESGCTDTETDITSMISRPASSQVSYEMGEDTTQTSDLGGKPKVKSHDSGIFRKTVVDADEIPMVEINDTEHSATSTCKTSEKCNVEEIQRSESLSGIGLREGESRHRTSASQIPSIIITYSNVQGVELPSGYSAGFLHPKNKSHKQNKSSNS

SEQ ID NO: 31 - protein, 357 aa, Gallus gallus
MSGMASDCNSSSQEEYLPHYVQQEDPFASKLSREADIIAGFYLTVIGILSTLGNGYVIFMSSKRKKKLRPAEIMTVNLAVCDLGISVVGKPFSIISFFSHRWIFGWMGCRWYGWAGFFFGCGSLITMTAVSLDRYLKICHLAYGTWLKRHHAFICLALIWAYATFWATVPFAGVGSYAPEPFGTSCTLDWWLAQASVAGQAFVLSILFFCLLFPTAVIVFSYVKIILKVKSSTKEVAHYDTRIQNSHILEMKLTKVAMLICAGFLIAWIPYAVVSVWSAFGQPDSVPIQFSVVPTLLAKSAAMYNPIIYQVIDCKFACCRSGGPKTLQKKSSLKESRMYTLSSHRDSAALSGTQLEV

SEQ ID NO: 32 - protein, 348 aa, Gallus gallus
MEEQYISKLHPVVDYGAGVFLLIIAILTILGNSAVLATAVKRSSLLKSPELLTVNLAVADIGMAISMYPLAIASAWNHAWLGGDASCIYYALMGFLFGVCSMMTLCAMAVIRFLVTNSSKSNSNKISKNTVHILITFIWLYSLLWAILPLVGWGYYGPEPFGISCTIAWSKFHSSSNGFSFILSMFLLCTVLPALTIVACYLGIAWKVHKAYQEIQNINRIPHAAKLEKKLTLMAVLISVGFLSAWTPYAAASFWSIFNSSDSLQPIVTLLPCLFAKSSTAYNPFIYYIFSKTFRHEIKQLQCCWGWRVHFFSADNSAENSVSMMWSGRDNIRLSPTAKVESQGAARH

SEQ ID NO: 33 - protein, 334 aa, Gallus gallus
MHWNDSANSSESDAEAHSVFTQTEHNIVAAYLITAGVISIFSNIVVLGIFVKYKEFRTATNAIIINLAFTDIGVSGIGYPMSAASDLHGSWKFGYTGCQIYAALNIFFGMASIGLLTVVAVDRYLTICRPDIGRRMTTRNYAALILAAWINAVFWASMPTVGWAGYASDPTGATCTANWRKNDVPFVSYTMSVIAVNFVVPLTVMFYCYYNVSRTMKQYTSSNCLESINMDWSDQVDVTKMSVVMIVMFLVAWSPYSIVCLWSSFGDPKKISPAMAIIAPLFAKSSTFYNPCIYVIANKKFRRAILAMVRCQTRQEITISNALPMTVSLSALTS

SEQ ID NO: 34 - protein, 295 aa, Gallus gallus
MVTSHPLPEGFTEIEVFAIGTALLVEALLGFCLNGLTIISFRKIKELRTPSNLLVLSIALADCGICINAFIAAFSSFLRYWPYGSEGCQIHGFQGFLTALASISSSAAVAWDRYHHYCTRSKLQWSTAISMMVFAWLFAAFWATMPLLGWGEYDYEPLRTCCTLDYSKGDRNYITFLFALSIFNFMIPGFIMMTAYQSIHQKFKKSGHYKFNTGLPLKTLVICWGPYCLLSFYAAIENVMFISPKYRMIPAIIAKTVPTVDSFVYALGNENYRGGIWQFLTGQKIEKAEVDSKTK

SEQ ID NO: 35 - DNA, 1047 bp, Homo sapiens
  source 1..1047: mol_type = genomic DNA
atgaatggcacagaaggccctaacttctacgtgcccttctccaatgcgacgggtgtggtacgcagccccttcgagtacccacagtactacctggctgagccatggcagttctccatgctggccgcctacatgtttctgctgatcgtgctgggcttccccatcaacttcctcacgctctacgtcaccgtccagcacaagaagctgcgcacgcctctcaactacatcctgctcaacctagccgtggctgacctcttcatggtcctaggtggcttcaccagcaccctctacacctctctgcatggatacttcgtcttcgggcccacaggatgcaatttggagggcttctttgccaccctgggcggtgaaattgccctgtggtccttggtggtcctggccatcgagcggtacgtggtggtgtgtaagcccatgagcaacttccgcttcggggagaaccatgccatcatgggcgttgccttcacctgggtcatggcgctggcctgcgccgcacccccactcgccggctggtccaggtacatccccgagggcctgcagtgctcgtgtggaatcgactactacacgctcaagccggaggtcaacaacgagtcttttgtcatctacatgttcgtggtccacttcaccatccccatgattatcatctttttctgctatgggcagctcgtcttcaccgtcaaggaggccgctgcccagcagcaggagtcagccaccacacagaaggcagagaaggaggtcacccgcatggtcatcatcatggtcatcgctttcctgatctgctgggtgccctacgccagcgtggcattctacatcttcacccaccagggctccaacttcggtcccatcttcatgaccatcccagcgttctttgccaagagcgccgccatctacaaccctgtcatctatatcatgatgaacaagcagttccggaactgcatgctcaccaccatctgctgcggcaagaacccactgggtgacgatgaggcctctgctaccgtgtccaagacggagacgagccaggtggccccggcctaa

SEQ ID NO: 36 - DNA, 1047 bp, Mus musculus
  source 1..1047: mol_type = genomic DNA
atgaacggcacagagggccccaatttttatgtgcccttctccaacgtcacaggcgtggtgcggagccccttcgagcagccgcagtactacctggcggaaccatggcagttctccatgctggcagcgtacatgttcctgctcatcgtgctgggcttccccatcaacttcctcacgctctacgtcaccgtacagcacaagaagctgcgcacacccctcaactacatcctgctcaacttggccgtggctgacctcttcatggtcttcggaggattcaccaccaccctctacacatcactccatggctacttcgtctttgggcccacaggctgtaatctcgagggcttctttgccacacttggaggtgaaatcgccctgtggtccctggtggtcctggccattgagcgctacgtggtggtctgcaagccgatgagcaacttccgcttcggggagaatcacgctatcatgggtgtggtcttcacctggatcatggcgttggcctgtgctgctcccccactcgttggctggtccaggtacatccctgagggcatgcaatgttcatgcgggattgactactacacactcaagcctgaggtcaacaacgaatcctttgtcatctacatgttcgtggtccacttcaccattcctatgatcgtcatcttcttctgctatgggcagctggtcttcacagtcaaggaggcggctgcccagcagcaggagtcagccaccactcagaaggcagagaaggaagtcacccgcatggttatcatcatggtcatcttcttcctgatctgctggcttccctacgccagtgtggccttctacatcttcacccaccagggctccaacttcggccccatcttcatgactctgccagctttctttgctaagagctcttccatctataacccggtcatctacatcatgttgaacaagcagttccggaactgtatgctcaccacgctgtgctgcggcaagaatccactgggagatgacgacgcctctgccaccgcttccaagacggagaccagccaggtggctccagcctaa

SEQ ID NO: 37 - DNA, 1047 bp, Canis familiaris
  source 1..1047: mol_type = genomic DNA
atgaacgggacggagggcccgaacttctacgtgcccttctccaacaagacgggtgtggtgcgcagccccttcgagtacccacagtactacctggctgagccatggcagttctccatgctggctgcctacatgtttctgctgatcgtgctcggcttccccatcaacttcctcacgctctacgtcacagtccagcacaagaagctgcgtacacctctcaactacatcctgctcaacctggctgtggctgacctcttcatggtcttcggtggcttcaccaccaccctctacacctctctgcatggatactttgtcttcgggcccacaggatgcaatgtggagggcttctttgccacactgggcggtgaaattgccctgtggtctttggtggtcctggccattgagcggtacgtggtggtgtgtaagcccatgagcaacttccgttttggggagaaccatgccatcatgggcgtcgccttcacctgggtcatggcgctggcctgtgcggcaccccccctcgctggctggtccaggtacatcccagagggcatgcagtgctcatgtgggatcgactactacacactcaagccagaaatcaacaatgagtccttcgtcatctacatgttcgtggtccacttcgccatccccatgattgtcatattcttctgctatggacagctcgtcttcacagtcaaggaggcagctgcccagcagcaggaatcggccaccacccagaaggctgaaaaggaggtcacccgcatggtcatcatcatggtcatcgctttcctgatctgctgggtgccctatgccagtgtggcattctacatcttcacccaccagggctccgactttggccccatcttcatgaccctcccagcgttcttcgccaagtcctcctccatctacaaccctgtcatctatatcatgatgaacaagcagttccggaactgcatgatcaccaccctctgctgcggcaagaacccactgggtgacgacgaggcctctgccagcgcctccaagacggagaccagccaggtggcaccggcctaa

SEQ ID NO: 38 - DNA, 1056 bp, Gallus gallus
  source 1..1056: mol_type = genomic DNA
atgaacgggacggaaggccaagacttctacgtgcccatgtccaacaagaccggggtggtgcggagccccttcgagtacccccagtactacctggctgagccctggaagttctcggcgctggctgcctacatgttcatgctgatcctgctcggcttccccgtcaacttcctcacgctgtacgtcaccatccagcacaagaaactccggacgcctctaaactacatcctcctgaacctggcggtcgccgacctctttatggtcttcggaggcttcacgaccaccatgtacacctcgatgaacgggtactttgtctttggagtaacagggtgctacatcgagggcttctttgctacgctgggcggtgaaattgctctctggtcactcgtcgtcctggccgtggaacgatacgtggtggtctgtaagcccatgagcaacttccgcttcggggagaaccacgccatcatgggggtcgcgttctcctggatcatggccatggcctgcgcagcccccccgctgttcggctggtcacggtacatccccgagggcatgcagtgctcgtgtgggatcgactactacacgctgaagccggagatcaacaacgaatcctttgtcatctacatgttcgtggtccacttcatgatcccactggccgtcatcttcttctgctatgggaacctggtctgcactgtgaaggaggctgccgcccagcagcaggagtctgccaccacccagaaggcagagaaggaagtgacccgcatggtgatcatcatggtcatcgccttcctcatctgctgggttccctacgccagcgtcgctttctacatcttcaccaaccagggctcagactttggacccatcttcatgaccatcccggcattctttgccaagagctctgccatctacaatcctgtgatctacatcgtaatgaacaaacagttccgtaactgcatgatcacaaccctctgctgcggcaagaacccgctgggcgatgaggacacgtctgctggaaagacagagacctcctccgtctccaccagccaggtgtcccctgcatag

SEQ ID NO: 39 - DNA, 1065 bp, Oryzias latipes
  source 1..1065: mol_type = genomic DNA
atgaatggcacagagggaccatatttttatgtccctatggtgaacaccaccggcattgtccggagtccttatgaatatcctcagtattaccttgtcaacccagcagcctatgctgctctgggcgcctacatgttttttctcatcctggttggcttccccatcaacttcctcactctctacgtcaccctcgaacacaagaagctgcgaacccctctaaactacatcctgctaaacctcgcggtggccgacctcttcatggtgttcggaggattcactacaacgatgtacacctccatgcacggctactttgtccttggacgtctcggctgcaatctggaaggattctttgctacccttggtggtgaaattggtctctggtcactggttgtcctggctattgagagatgggttgttgtctgcaagcccatcagcaacttccgctttggtgagaatcatgctattatgggtttggtcttcacctggatcatggctgcctcctgtgccgtgccccctctcgtcggctggtctcgttacatcccagagggcatgcagtgctcatgtggagtcgactactacacccgtgcagagggcttcaacaatgagtcctttgttgtctacatgttcgtctgccacttcctaattccactgatcgttgtgttcttctgctacggccgtctgctctgtgctgtcaaggaggctgctgctgcccagcaggagtctgagaccacccagagagctgagagggaagtcacccgcatggttgtcatcatggtcatcggcttcctggtatgttggcttccctatgccagtgtggcctggtacatcttcacaaatcagggctctgaattcgggccactcttcatgaccatcccagccttctttgccaagagttcttccatctacaacccagcaatctacatctgcatgaacaagcagttccgcaactgcatgatcaccaccctgtgctgtgggaagaatccctttgaagaggaggagggagcctccactactgcttccaagaccgaggcctcatctgtctcctcaagctctgtgtcccctgcataa

SEQ ID NO: 40 - DNA, 1047 bp, Homo sapiens
  source 1..1047: mol_type = genomic DNA
atgagaaaaatgtcggaggaagagttttatctgttcaaaaatatctcttcagtggggccgtgggatgggcctcagtaccacattgcccctgtctgggccttctacctccaggcagctttcatgggcactgtcttccttatagggttcccactcaatgccatggtgctggtggccacactgcgctacaaaaagttgcggcagcccctcaactacattctggtcaacgtgtccttcggaggcttcctcctctgcatcttctctgtcttccctgtcttcgtcgccagctgtaacggatacttcgtcttcggtcgccatgtttgtgctttggagggcttcctgggcactgtagcaggtctggttacaggatggtcactggccttcctggcctttgagcgctacattgtcatctgtaagcccttcggcaacttccgcttcagctccaagcatgcactgacggtggtcctggctacctggaccattggtattggcgtctccatcccacccttctttggctggagccggttcatccctgagggcctgcagtgttcctgtggccctgactggtacaccgtgggcaccaaataccgcagcgagtcctatacgtggttcctcttcatcttctgcttcattgtgcctctctccctcatctgcttctcctacactcagctgctgagggccctgaaagctgttgcagctcagcagcaggagtcagctacgacccagaaggctgaacgggaggtgagccgcatggtggttgtgatggtaggatccttctgtgtctgctacgtgccctacgcggccttcgccatgtacatggtcaacaaccgtaaccatgggctggacttacggcttgtcaccattccttcattcttctccaagagtgcttgcatctacaatcccatcatctactgcttcatgaataagcagttccaagcttgcatcatgaagatggtgtgtgggaaggccatgacagatgaatccgacacatgcagctcccagaaaacagaagtttctactgtctcgtctacccaagttggccccaactga

SEQ ID NO: 41 - DNA, 1095 bp, Homo sapiens
  source 1..1095: mol_type = genomic DNA
atggcccagcagtggagcctccaaaggctcgcaggccgccatccgcaggacagctatgaggacagcacccagtccagcatcttcacctacaccaacagcaactccaccagaggccccttcgaaggcccgaattaccacatcgctcccagatgggtgtaccacctcaccagtgtctggatgatctttgtggtcactgcatccgtcttcacaaatgggcttgtgctggcggccaccatgaagttcaagaagctgcgccacccgctgaactggatcctggtgaacctggcggtcgctgacctagcagagaccgtcatcgccagcactatcagcattgtgaaccaggtctctggctacttcgtgctgggccaccctatgtgtgtcctggagggctacaccgtctccctgtgtgggatcacaggtctctggtctctggccatcatttcctgggagagatggatggtggtctgcaagccctttggcaatgtgagatttgatgccaagctggccatcgtgggcattgccttctcctggatctgggctgctgtgtggacagccccgcccatctttggttggagcaggtactggccccacggcctgaagacttcatgcggcccagacgtgttcagcggcagctcgtaccccggggtgcagtcttacatgattgtcctcatggtcacctgctgcatcatcccactcgctatcatcatgctctgctacctccaagtgtggctggccatccgagcggtggcaaagcagcagaaagagtctgaatccacccagaaggcagagaaggaagtgacgcgcatggtggtggtgatgatctttgcgtactgcgtctgctggggaccctacaccttcttcgcatgctttgctgctgccaaccctggttacgccttccaccctttgatggctgccctgccggcctactttgccaaaagtgccactatctacaaccccgttatctatgtctttatgaaccggcagtttcgaaactgcatcttgcagcttttcgggaagaaggttgacgatggctctgaactctccagcgcctccaaaacggaggtctcatctgtgtcctcggtatcgcctgcatga

SEQ ID NO: 42 - DNA, 1095 bp, Homo sapiens
  source 1..1095: mol_type = genomic DNA
atggcccagcagtggagcctccaaaggctcgcaggccgccatccgcaggacagctatgaggacagcacccagtccagcatcttcacctacaccaacagcaactccaccagaggccccttcgaaggcccgaattaccacatcgctcccagatgggtgtaccacctcaccagtgtctggatgatctttgtggtcattgcatccgtcttcacaaatgggcttgtgctggcggccaccatgaagttcaagaagctgcgccacccgctgaactggatcctggtgaacctggcggtcgctgacctggcagagaccgtcatcgccagcactatcagcgttgtgaaccaggtctatggctacttcgtgctgggccaccctatgtgtgtcctggagggctacaccgtctccctgtgtgggatcacaggtctctggtctctggccatcatttcctgggagagatggatggtggtctgcaagccctttggcaatgtgagatttgatgccaagctggccatcgtgggcattgccttctcctggatctgggctgctgtgtggacagccccgcccatctttggttggagcaggtactggccccacggcctgaagacttcatgcggcccagacgtgttcagcggcagctcgtaccccggggtgcagtcttacatgattgtcctcatggtcacctgctgcatcaccccactcagcatcatcgtgctctgctacctccaagtgtggctggccatccgagcggtggcaaagcagcagaaagagtctgaatccacccagaaggcagagaaggaagtgacgcgcatggtggtggtgatggtcctggcattctgcttctgctggggaccatacgccttcttcgcatgctttgctgctgccaaccctggctaccccttccaccctttgatggctgccctgccggccttctttgccaaaagtgccactatctacaaccccgttatctatgtctttatgaaccggcagtttcgaaactgcatcttgcagcttttcgggaagaaggttgacgatggctctgaactctccagcgcctccaaaacggaggtctcatctgtgtcctcggtatcgcctgcatga

SEQ ID NO: 43 - DNA, 1041 bp, Mus musculus
  source 1..1041: mol_type = genomic DNA
atgtcaggagaggatgacttttacctgtttcagaatatctcttcggtggggccctgggatgggcctcagtaccaccttgctcctgtctgggccttccgcctccaggcagccttcatgggatttgtcttctttgtggggaccccactcaatgccatagtgctggtggccacactgcattacaaaaagttgcgacagcccctcaactatattctggtcaatgtatccctcgggggcttcctcttctgcatcttctctgtcttcacagtcttcatcgccagctgtcacggatacttcctctttggtcgccatgtttgtgctctggaggccttcttgggctctgtagcaggtctagtgacaggatggtcattggctttcctggcttttgaacgctacgttgtcatctgtaaacccttcggcagcatccgcttcaactccaagcatgcactgatggtggtcctggctacttggattattggtatcggggtgtccatcccacccttttttggctggagcaggttcatccctgagggcctgcagtgctcctgtggcccagactggtacactgtgggcaccaagtatcgaagcgagtactacacctggttcctcttcatcttctgtttcatcattcctctttccctcatctgcttctcctactcccagttgctgaggactctcagagctgtggcagctcagcagcaagagtctgctacgacacaaaaggctgaacgggaggtgagtcatatggtggtggtgatggtgggatccttctgtctctgctacgtgccctatgctgccctggccatgtacatggtcaacaatcggaaccacgggctggacttacggcttgtcaccatccccgccttcttttccaagagctcctgtgtctacaaccccatcatctactgcttcatgaataagcagttccgggcttgcattctggagatggtgtgcaggaagcccatggcagacgaatctgacgtgtctggctctcagaaaacagaagtttctactgtctcttctagcaaagttggccctcactga

SEQ ID NO: 44 - DNA, 1080 bp, Mus musculus
  source 1..1080: mol_type = genomic DNA
atggcccaaaggcttacaggtgaacagacactggaccactatgaggatagcacccatgcaagcatcttcacctataccaacagcaacagcaccaaaggtccctttgaaggccccaattatcacattgctcccaggtgggtgtaccacctcaccagcacctggatgattcttgtggtcgttgcatctgtcttcactaatggacttgtgctggcagccaccatgagattcaagaagctgcgccatccactgaactggattctggtgaacttggcagttgctgacctagcagagaccattattgccagcactatcagtgttgtgaaccaaatctatggctacttcgttctgggacaccctctgtgtgtcattgaaggctacattgtctcattgtgtggaatcacaggcctctggtccctggccatcatttcctgggagagatggctggtggtctgcaagccctttggcaatgtgagatttgatgctaagctggccactgtgggaatcgtcttctcctgggtctgggctgctatatggacggccccaccaatctttggttggagcaggtactggccttatggcctgaagacatcctgtggcccagacgtgttcagcggtacctcgtaccccggggttcagtcttatatgatggtcctcatggtcacgtgctgcatcttcccactcagcatcatcgtgctctgctacctccaagtgtggctggccatccgagcagtggcaaagcaacagaaagaatctgagtccactcagaaggccgagaaggaggtgacacgcatggtggtggtgatggtcttcgcatactgcctctgctggggaccctatactttctttgcatgctttgctactgcccaccctggctatgccttccaccctcttgtggcctccctaccatcctactttgccaaaagtgccactatctacaaccccattatctatgtctttatgaaccggcagtttcgaaactgcatcttacatctctttggaaagaaggttgatgatagctctgaactttccagcacctccaagacagaagtctcatctgtctcttcagtgtcacctgcataa

SEQ ID NO: 45 - DNA, 1068 bp, Gallus gallus
  source 1..1068: mol_type = genomic DNA
atgaatgggacagaaggtatcaatttttatgtgcctatgtccaacaagacaggggtggtgcgaagccccttcgagtacccccagtattacctagccgagccctggaaataccgccttgtgtgttgctacatcttcttcctcatctccactggtctgcccatcaacctcctcaccctcctggtcaccttcaaacacaagaagctccggcagccgctcaactacatcctggtcaacctggcggtggctgacctcttcatggcctgcttcggcttcaccgtcactttctacacagcctggaatggatatttcgtcttcggtcccgttggctgtgctgtggagggcttcttcgccactctgggaggccaggttgccctctggtccctggtggtcttggccatagagcgttacatcgttgtctgcaagcccatgggaaacttccgcttctctgccacccacgccatgatgggcatagctttcacctgggtcatggccttctcctgtgctgctccacccctctttggctggtccaggtacatgccggaggggatgcagtgctcctgtggccctgactattacacccacaaccctgactaccacaacgagtcctacgtcctctacatgtttgtcatccacttcatcatcccggtcgtggtcatcttcttctcctatgggcgcctcatctgcaaagtccgagaggcagccgcgcagcagcaggagtcagccaccacccagaaggcagagaaggaggtgacgcggatggtgatcctgatggtgctgggcttcatgctggcctggacaccctatgctgtagtggcattctggatcttcaccaacaagggagcagacttcaccgccacactgatggcagtgcctgccttcttctccaagagctcctctctctacaaccccatcatctatgtcctcatgaacaagcagttccgtaattgcatgatcaccactatctgctgtggcaagaacccttttggtgacgaagatgtctcttccaccgtatcccagagcaagactgaggtctcctctgtctcctccagccaagtttcacctgcatag

SEQ ID NO: 46 - DNA, 1086 bp, Gallus gallus
  source 1..1086: mol_type = genomic DNA
atgcaccccccccgccccaccacggacctcccggaggatttctacatccccatggctttggacgcccccaacattacggcgctcagccccttcctggtcccccaaacccacctgggcagcccggggctgttcagagctatggcggcctttatgttcctcctcatcgctttgggggtccccatcaacacgttgaccattttttgcaccgcccgtttccggaagctccgttcccaccttaattacatcctggttaatttggccttggccaacctgctggtgatcctggtgggctccaccacggcctgttacagcttctcgcagatgtacttcgccctcggacccacggcgtgcaaaatcgagggcttcgctgccacgctgggaggcatggtgagtctgtggtcgttggccgtggtggcgttcgagcgcttcctcgtcatctgcaaacctttgggcaacttcacgttccgcggcagccacgccgtgttgggctgcgtggccacgtgggtgctcggattcgtcgcctccgcgccgccgctcttcggatggagtcggtacatcccggaggggctgcagtgctcgtgcgggccggactggtacacgacggacaacaagtggcacaacgagagctacgtgctcttcctgttcaccttctgcttcggggtccctctcgccatcatcgtcttctcctacggccgcctcctcatcacactcagagcggttgcccggcagcaggagcagtcagcgacgacgcagaaggcggaccgggaggtgacgaagatggtggtggtgatggtgctgggcttcctggtgtgctgggcgccatacacggccttcgcgctgtgggtggtgacgcaccgcgggcgcagcttcgaggtgggattggcctccatcccctccgtcttctccaagtcctccaccgtctacaaccccgtcatctacgtcctcatgaacaagcagttccgctcgtgcatgctgaagctgctgttctgcggccgcagtccgttcggggacgacgaggacgtgtcgggctcctcgcaggccacgcaggtctcctccgtctcctccagccacgtcgcccccgcctaa

SEQ ID NO: 47 - DNA, 1044 bp, Gallus gallus
  source 1..1044: mol_type = genomic DNA
atgtcatcggacgacgacttctacctcttcaccaacggctcagtgccgggcccgtgggacggcccccaataccacatcgcccccccgtgggccttctacctacagacggccttcatggggatcgtattcgccgtggggaccccactgaacgccgtggtgctgtgggtcaccgttcgttacaaacgactccggcagccccttaattacatcctggtcaacatctcggccagcggattcgtctcctgcgtgctcagcgtcttcgtcgtcttcgtggccagcgcccgcggatacttcgtcttcgggaagagggtctgcgagttggaggccttcgtgggcacccacggggggctggtgacgggatggtccctggcctttttggccttcgagcgttacatcgttatctgcaaaccgttcggcaacttccggttcagctcccggcacgccctgctggtcgtcgtggccacgtggctcatcggcgtcggcgtcggactgccccccttcttcgggtggagccggtacatgcctgagggtctgcagtgctcgtgtggccccgactggtacacggtgggcacgaaataccgcagcgagtactacacgtggttcctcttcatcttctgcttcatcgtccccctctccctcatcatcttctcctactcccaactgctgagcgccctgcgagccgtggcggcgcagcagcaggagtcggccacgacgcagaaggcggagcgggaggtgtcgcggatggtggtggtgatggtggggtcgttctgcctctgctacgtcccctacgccgccctcgccatgtatatggtcaacaaccgcgaccacggcttggacctccgcctcgtcaccatccccgccttcttctccaagagcgcctgcgtctacaaccccatcatctactgcttcatgaacaagcagttccgcgcctgcatcatggagacggtttgcgggaagccgctgacggacgattcggacgcgtcgacttcagcgcagaggacggaggtgtcctccgtgtcctccagccaagtcggccccacttag

SEQ ID NO: 48 - DNA, 1089 bp, Gallus gallus
  source 1..1089: mol_type = genomic DNA
atggcggcgtgggaggcggcgttcgccgctcggaggcggcacgaagaggaggacaccacgcgcgacagcgtcttcacctacaccaacagcaacaacacccgcggaccatttgagggccccaactaccacatagcgccgcgctgggtgtacaacctgacgtcgctgtggatgatcttcgtggtggcggcgtcggtgttcaccaacgggttggtgctcgtggccacctggaagttcaagaagctgcgccaccccctcaactggatcctggtgaacctcgccgtggccgacctgggcgagaccgtcatcgcctccaccatcagcgtcatcaaccagatctcggggtacttcatcctcgggcaccccatgtgcgtcgtcgagggatacaccgtgtctgcatgcggcattacggcgctgtggtcgctggcgatcatttcgtgggagcggtggttcgtggtgtgcaaaccgttcgggaacatcaaattcgacgggaagttggcggtggcgggaatcctcttctcctggctgtggtcctgcgcgtggaccgcgccgcccatcttcgggtggagccggtattggccccacggcctgaagacgtcgtgcggcccggatgtgttcagcggcagctccgacccgggggtgcagtcctacatggtggtgctgatggtcacgtgctgcttcttccccctcgccatcatcatcctctgctacctgcaagtctcgctcgccatccgcgccgtggcggctcagcagaaggagtcggagtcgacgcagaaggcggagaaggaggtgtcccgcatggtggtggtgatgatcgtggcctactgcttctgctgggggccctacaccttcttcgcctgcttcgccgccgccaaccccggctacgccttccaccccctggcggccgccctgcccgcctacttcgccaagtcggccaccatctacaaccccatcatctacgtcttcatgaaccgacagttccggaactgcatcctgcagctcttcggcaaaaaggtggacgacggctccgaggtgtccacgtcgcgcacggaggtctcctccgtctccaactcctccgtctcgcccgcctaa

SEQ ID NO: 49 - DNA, 1056 bp, Gallus gallus
  source 1..1056: mol_type = genomic DNA
atgtcctccaacagctcccaggcacctcccaatgggaccccagggccttttgatggcccccagtggccctaccaggccccacagagcacatatgtgggggtggccgtgctgatgggcacggtggtcgcctgtgcctcggtggtgaatgggctggtcatcgtggtgtccatctgctacaaaaagctccgctccccactgaattacatcctggtgaacctggccgtggctgacctgctggtgacgctgtgcggcagctccgtcagcctctccaacaacatcaatggcttcttcgtgtttggcaggaggatgtgtgagctggagggcttcatggtctccttgacaggcatcgtggggctgtggtcgctggccatcctggccctggagcgctacgttgtggtctgcagacccctgggagatttccagttccaacgtcggcacgcggtgagcggctgcgccttcacgtggggctgggcgctgctctggagcaccccaccactgctgggctggagcagctacgtgcctgaagggttgaggacatcgtgcgggcctaactggtacacgggtggcagcaacaacaacagctacatcctgtccctgtttgtcacctgcttcgtcctgccgctcagcctcatcctcttctcctacacaaacctgctgctgaccctgcgggcggctgcagcacagcagaaggaagctgacaccacgcagcgggcggagcgggaggtgacgcggatggtgatcgtgatggtgatggccttcctgctctgctggctgccctacagcacgtttgccttggtggtggccacccataagggcatcatcatccagccggtcctcgcctccttgccttcctatttctccaagacagccaccgtgtacaatcccatcatctacgtcttcatgaacaaacagttccagagctgcctgctggaaatgctgtgctgtggttaccagccccagcggacaggaaaagcctcaccggggacacctgggccccatgcagatgtcactgcagcggggctgaggaacaaggtgatgccagcacaccccgtgtga

SEQ ID NO: 50 - DNA, 1209 bp, Homo sapiens
  source 1..1209: mol_type = genomic DNA
atgtactcggggaaccgcagcggcggccacggctactgggacggcggcggggccgcgggcgctgaggggccggcgccggcggggacactgagccccgcgcccctcttcagccccggcacctacgagcgcctggcgctgctgctgggctccattgggctgctgggcgtcggcaacaacctgctggtgctcgtcctctactacaagttccagcggctccgcactcccactcacctcctcctggtcaacatcagcctcagcgacctgctggtgtccctcttcggggtcacctttaccttcgtgtcctgcctgaggaacggctgggtgtgggacaccgtgggctgcgtgtgggacgggtttagcggcagcctcttcgggattgtttccattgccaccctaaccgtgctggcctatgaacgttacattcgcgtggtccatgccagagtgatcaatttttcctgggcctggagggccattacctacatctggctctactcactggcgtgggcaggagcacctctcctgggatggaacaggtacatcctggacgtacacggactaggctgcactgtggactggaaatccaaggatgccaacgattcctcctttgtgcttttcttatttcttggctgcctggtggtgcccctgggtgtcatagcccattgctatggccatattctatattccattcgaatgcttcgttgtgtggaagatcttcagacaattcaagtgatcaagattttaaaatatgaaaagaaactggccaaaatgtgctttttaatgatattcaccttcctggtctgttggatgccttatatcgtgatctgcttcttggtggttaatggtcatggtcacctggtcactccaacaatatctattgtttcgtacctctttgctaaatcgaacactgtatacaatccagtgatttatgtcttcatgatcagaaagtttcgaagatcccttttgcagcttctgtgcctccgactgctgaggtgccagaggcctgctaaagacctaccagcagctggaagtgaaatgcagatcagacccattgtgatgtcacagaaagatggggacaggccaaagaaaaaagtgactttcaactcttcttccatcatttttatcatcaccagtgatgaatcactgtcagttgacgacagcgacaaaaccaatgggtccaaagttgatgtaatccaagttcgtcctttgtag

SEQ ID NO: 51 - DNA, 1437 bp, Homo sapiens
  source 1..1437: mol_type = genomic DNA
atgaaccctccttcggggccaagagtcctgcccagcccaacccaagagcccagctgcatggccaccccagcaccacccagctggtgggacagctcccagagcagcatctccagcctgggccggcttccatccatcagtcccacagcacctgggacttgggctgctgcctgggtccccctccccacggttgatgttccagaccatgcccactataccctgggcacagtgatcttgctggtgggactcacggggatgctgggcaacctgacggtcatctataccttctgcaggagcagaagcctccggacacctgccaacatgttcattatcaacctcgcggtcagcgacttcctcatgtccttcacccaggcccctgtcttcttcaccagtagcctctataagcagtggctctttggggagacaggctgcgagttctatgccttctgtggagctctctttggcatttcctccatgatcaccctgacggccatcgccctggaccgctacctggtaatcacacgcccgctggccacctttggtgtggcgtccaagaggcgtgcggcatttgtcctgctgggcgtttggctctatgccctggcctggagtctgccacccttcttcggctggagcgcctacgtgcccgaggggttgctgacatcctgctcctgggactacatgagcttcacgccggccgtgcgtgcctacaccatgcttctctgctgcttcgtgttcttcctccctctgcttatcatcatctactgctacatcttcatcttcagggccatccgggagacaggacgggctctccagaccttcggggcctgcaagggcaatggcgagtccctgtggcagcggcagcggctgcagagcgagtgcaagatggccaagatcatgctgctggtcatcctcctcttcgtgctctcctgggctccctattccgctgtggccctggtggcctttgctgggtacgcacacgtcctgacaccctacatgagctcggtgccagccgtcatcgccaaggcctctgcaatccacaaccccatcatttacgccatcacccaccccaagtacagggtggccattgcccagcacctgccctgcctgggggtgctgctgggtgtatcacgccggcacagtcgcccctaccccagctaccgctccacccaccgctccacgctgaccagccacacctccaacctcagctggatctccatacggaggcgccaggagtccctgggctcggagagtgaggtgggctggacacacatggaggcagcagctgtgtggggagctgcccagcaagcaaatgggcggtccctctacggtcagggtctggaggacttggaagccaaggcaccccccagaccccagggacacgaagcagagactccagggaagaccaaggggctgatccccagccaggaccccaggatgtag

SEQ ID NO: 52 - DNA, 1065 bp, Homo sapiens
  source 1..1065: mol_type = genomic DNA
atggcgttaaatcacactgccctgcctcaggacgagcgcctgccccattaccttcgagatggggatccttttgcttccaaactttcttgggaagcggatttagtggctggcttttacctaacaataattgggattctgtccacatttggaaatggatatgtcctttacatgtcttctagacgaaagaagaagctgagacccgctgaaataatgactatcaatttagcagtctgtgatctggggatttcagttgtaggcaagccgttcaccatcatctcttgcttttgtcaccgctgggtgtttggctggatcggctgccgctggtatggatgggctggatttttctttggctgtggaagccttatcaccatgactgctgtcagcctggatcgatatttgaaaatctgctatttatcttatggggtttggctgaaaagaaagcacgcctacatctgcctggcagccatctgggcctatgcttccttctggaccaccatgcccttggtaggtctgggggactacgtacctgagcccttcggaacctcgtgcaccctggactggtggctggcccaggcctcggtagggggccaggttttcatcctgaacatcctcttcttctgcctcttgctcccaacggctgtgatcgtgttctcctacgtaaagatcattgccaaggttaagtcctcttccaaagaagtagctcatttcgacagtcggatccatagcagccatgtgctggaaatgaaactgacaaaggtagcgatgttgatttgtgctggattcctgattgcctggattccttatgcagtggtgtctgtgtggtcagcttttggaaggccagactccattcccatacagctctctgtggtgccaaccctacttgcaaaatctgcagcgatgtacaatcccatcatttaccaagttattgattacaaatttgcctgttgccaaactggtggtttgaaagcaaccaagaagaagtctctggaaggcttcaggctgcacaccgtaaccacagtcaggaagtcttctgctgtgctggaaattcatgaagagtgggaataa

SEQ ID NO: 53 - DNA, 876 bp, Homo sapiens
  source 1..876: mol_type = genomic DNA
atggcagagaccagtgccctgcccactggcttcggggagctcgaggtgctggctgtggggatggtgctactggtggaagctctctccggtctcagcctcaataccctgaccatcttctctttctgcaagaccccggagctgcggactccctgccacctactggtgctgagcttggctcttgcggacagtgggatcagcctgaatgccctcgttgcagccacatccagccttctccggcgctggccctacggctcggacggctgccaggctcacggcttccagggctttgtgacagcgttggccagcatctgcagcagtgcagccatcgcatgggggcgttatcaccactactgcacccgtagccagctggcctggaactcagccgtctctctggtgctcttcgtgtggctgtcttctgccttctgggcagctctgccccttctgggttggggtcactatgactatgagccactggggacatgctgcaccctggactactccaagggggacagaaacttcaccagcttcctcttcaccatgtccttcttcaacttcgccatgcccctcttcatcacgatcacttcctacagtctcatggagcagaaactggggaagagtggccatctccaggtaaacaccactctgccagcaaggacgctgctgctcggctggggcccctatgccatcctgtatctatacgcagtcatcgcagacgtgacttccatctcccccaaactgcagatggtgcccgccctcattgccaaaatggtgcccacgatcaatgccatcaactatgccctgggcaatgagatggtctgcaggggaatctggcagtgcctctcaccgcagaagagggagaaggaccgaaccaagtga

SEQ ID NO: 54 - DNA, 1014 bp, Homo sapiens
  source 1..1014: mol_type = genomic DNA
atgctaagaaataatttaggcaacagttcagactctaaaaatgaagatggctcggtcttttcacagactgaacacaatattgttgcaacttacttgattatggcaggtatgataagtattatcagcaacataatagttctgggcatcttcattaagtacaaggaacttcggacacccacaaatgcaattattattaacctggctgttactgatataggggtcagtagcattggctatcccatgtctgctgcctcagatctgtatggaagttggaaatttggatacgcaggctgtcaggtttatgctggattgaatattttttttggaatggcaagcattggattactcacggtcgtggctgtggaccgatacctgaccatctgccttcctgacgtagggagaagaatgaccaccaacacttacatcggcttgattctgggagcctggatcaatggcctgttttgggctttgatgcctatcatagggtgggctagttatgccccagatcctactggtgctacgtgtaccataaactggaggaaaaatgatagatcttttgtgtcttacaccatgacagttattgcgataaattttattgtgcccttgacagtgatgttttactgctattaccatgtcacgctatccattaaacatcacactaccagtgactgcactgagtccctcaacagagactggtcagatcagatagatgtaacaaagatgtctgtgatcatgatctgcatgtttctggtggcatggtccccttattccatcgtgtgcttatgggcttcttttggtgacccaaagaagattcctccccccatggccatcatagctccactgtttgcaaaatcttctacattctataacccctgcatttatgtggttgctaataaaaagtttcggagggcaatgcttgccatgttcaaatgtcagactcaccaaacaatgcctgtgacaagtattttacccatggatgtatctcaaaacccattggcttctggaagaatctga

SEQ ID NO: 55 - DNA, 1203 bp, Mus musculus
  source 1..1203: mol_type = genomic DNA
atgtactcggggaaccgtagtggcgaccagggctactgggaggacggggcgggcgccgagggcgcagcaccggcgggcacgcggagccccgcgcctctcttcagccccaccgcgtacgagcgcctggcgctgctactcggctgcctcgcgctgctgggcgtcggcggcaacctgctggtgctgcttctctactccaagttcccgagactgcgcacgcccacccacctcttcctggtcaacctgagcctgggcgacctgctggtatccctgttcggagtcaccttcaccttcgcgtcgtgcctgcggaacggctgggtgtgggacgccgtgggctgcgcgtgggacgggtttagcggcagcctctttgggttcgtttccattaccaccctcactgtgctggcctatgaacgttatatccgtgtggtacatgccagagtgatcaacttttcctgggcctggagggccattacctatatctggctctactccttggcatgggcaggagcacctctcctgggctggaacaggtacatcctagacatacatggactgggctgtaccgtggactggagatccaaggatgccaacgactcttcctttgtgctcttcctgtttctcggctgcctggtggtgcccgtgggcatcatagcccattgctacggccacattctctattctgttcgaatgcttcgctgtgttgaagatcttcagaccattcaagtgatcaagatgctaagatatgaaaagaaagtagcaaagatgtgctttttgatggcctttgtctttctcacctgctggatgccttacattgtgacccgcttcttggtggtcaatggctatggacacctggtcaccccaactgtgtctattgtttcttatctctttgctaaatcgagcactgtgtacaacccagttatctacatcttcatgaacagaaagtttcggaggtcccttctgcagctcctatgcttccgcctgctgagatgccagcggcctgctaaaaacctcccagcggctgagagtgaaatgcacatcaggcccatcgtgatgtcacagaaagatggggacaggccaaagaagaaagtgacctttaactcttcctctatcatctttatcatcaccagtgatgagtccctgtcagtcgaggacagtgacagaagcagcgcatctaaggtcgatgtcatccaagtgcgtcctctataa

SEQ ID NO: 56 - DNA, 1566 bp, Mus musculus
  source 1..1566: mol_type = genomic DNA
atggactctccttcaggaccaagagtcttgtcaagcttaactcaggatcccagcttcacaaccagtcctgccctgcaaggcatttggaacggcactcagaacgtctccgtaagagcccagcttctctctgttagccccacgacatctgcacatcaggctgctgcctgggtccccttccccacagtcgatgtcccagaccatgctcactataccctaggcacggtgatcctgctggtgggactcacagggatgctgggcaatctgacggtcatctacaccttctgcaggaacagaggcctgcggacaccagcaaacatgttcatcatcaacctcgcagtcagcgacttcctcatgtcagtcactcaggccccggtcttctttgccagcagcctctacaagaagtggctctttggggagacaggttgcgagttctatgccttctgcggggctgtctttggcatcacttccatgatcaccctgacagccatagccatggaccgctatctggtgatcacacgtccactggccaccatcggcaggggatccaaaagacgaacggcactcgtcctgctaggcgtctggctttatgccctggcctggagtctgccacctttctttggttggagtgcctacgtgcccgaggggctgctgacatcctgctcctgggactacatgaccttcacaccccaggtgcgtgcctacaccatgctgctcttctgctttgtcttcttcctccccctgctcatcatcatcttctgctacatcttcatcttcagggccatccgagagacaggccgggcctgtgagggctgcggtgagtcccctctgcggcagaggcggcagtggcagcggctgcagagtgagtggaagatggccaaggtcgcactgattgtcattcttctcttcgtgctgtcctgggctccctactccactgtggctctggtggcctttgctggatactcgcacatcctgacgccctacatgagctcggtgccagccgtcatcgccaaggcttctgccatccacaatcccattatctacgccatcactcaccccaagtacagggtggccattgcccagcacctgccttgccttggggtgcttctcggtgtatcaggccagcgcagccacccctccctcagctaccgctctacccaccgctccacattgagcagccagtcctcagacctcagctggatctctggacggaagcgtcaagagtccctgggttctgagagtgaagtgggctggacagacacagaaacaaccgctgcatggggagctgcccagcaagcaagtggacagtccttctgcagtcagaacctagaagatggagaactcaaggcctcttccagcccccaggtacagagatctaagactcccaaggtgcctggacccagtacctgccgccctatgaaaggacagggagccaggccaagtagcctaaggggtgaccagaaaggcaggcttgctgtgtgcacaggcctctcagagtgtccccatccccatacatcccagtttccccttgctttcctagaggatgatgtgactctcagacatctgtag

SEQ ID NO: 57 - DNA, 1134 bp, Mus musculus
  source 1..1134: mol_type = genomic DNA
atggccttgaaccacactgccctacctcaggatgagcgcctgccccactatcttcgagacgaggacccttttgcttccaaactttcctgggaagcggatttagtggctggcttttacctaacaataatcgggattctctctacatttggaaatgggtatgtcctttatatgtcttctagacgcaagaagaagctgagacctgcggaaataatgactatcaatttagcagtctgtgatctggggatatcagttgtaggcaagccgttcaccatcatctcttgcttctgccaccgctgggtgtttggctggtttggctgccgctggtatggctgggctggatttttctttggctgtggaagcctgattaccatgactgctgtcagcctggaccgctatctgaagatctgttatctgtcttatggggtctggctgaagagaaagcatgcctacatctgcctggcagtcatctgggcttatgcttccttctggaccaccatgcccttggtgggcctgggggactatgcacctgagcccttcggaacctcatgcaccctggactggtggctggcccaggcttcaggtgggggtcaggtgttcatcctgagcatcctcttcttctgcctcctgctgccaacggctgtgattgttttctcatatgctaagatcatcgccaaggtgaagtcttcttctaaagaggtagcccatttcgacagtcgaatccatagcagccatgtacttgaggtgaagctgaccaaggtggcaatgctgatttgtgctggtttcctgattgcctggattccttatgcggtcgtctctgtgtggtcagcctttggaaggccagactccatccccatacagctctccgtggtgcccacactccttgcaaaatcagcagcgatgtacaatccaatcatctaccaggtcattgattacagatttgcctgttgccaggctggtggtttgagaggaacgaagaagaaatctttggaagactttaggctgcatactgtaaccgcagtcaggaagtcttctgctgtgctggagatccatccagagagcagttccagatttactagtgcccatgttatggatggagagagtcacagtaatgatggtgactgtggcaagaaataa

SEQ ID NO: 58 - DNA, 876 bp, Mus musculus
  source 1..876: mol_type = genomic DNA
atggcagcaaccagggccctgcctgctggtttgggggaacttgaggtgctggctgtaggaacagtcctgctgatggaagcgctctctggcatcagcctcaatggcctgaccatcttctctttctgcaagactccagatctgcggactcccagcaacctgctggtactgagcctggccctggcagacactgggatcagcctgaatgcccttgttgcagcggtatccagcctcctccggcgctggccacatggttcagagggctgccaggttcatggtttccagggatttgcaacagcactggccagcatctgtggcagtgcagccgttgcctggggacgttatcaccactactgcacccgcagacagttggcatgggacacggccatccctctggtgctgtttgtgtggatgtcatctgccttctgggcatccctgcccctgatgggctggggccactatgactatgagcctgtggggacatgctgtacactggactattcgaggggtgacagaaacttcatcagttttctcttcaccatggcttttttcaacttcctcgtacccctgttcatcacacacacttcataccggttcatggagcagaaattctccaggagtggccatctcccggtgaatactactcttccaggcagaatgctgctgcttggctggggcccctatgccctcctgtacctatacgcagccatcgcagatgtgagcttcatctctcctaaactacagatggtgcctgctctcatcgccaaaaccatgcccacaatcaacgccatcaactatgcgttgcacagggagatggtctgtagaggaacctggcagtgtctgtctccacaaaaaagcaagaaggaccgaacccagtga

SEQ ID NO: 59 - DNA, 1014 bp, Mus musculus
  source 1..1014: mol_type = genomic DNA
atgctgagtgaggcttcggattttaacagctcgggctctaggagcgaaggttctgtcttttcaaggactgagcacagcgtcatagcggcttacctgattgtggcaggtatcacgagcattctcagcaacgtagtagtcctgggtatcttcatcaagtacaaggagctgcggacacccaccaatgcagtgattatcaacctggctttcacggatataggggtcagtagcatcggctatcccatgtctgcggcttcagatctgcatggaagttggaaatttggacatgcaggctgtcagatttatgcaggactgaatatcttctttgggatggtgagcattggcttactcacggttgtagctatggatcggtacctgaccatcagttgccctgatgtaggacgaagaatgaccaccaacacttacctcagcatgatcctgggcgcctggatcaatggcctgttttgggctttgatgcccatcatagggtgggctagttatgccccggatcctacaggggccacgtgtaccataaactggcggaataatgatacctcgttcgtgtcttacaccatgatggttatcgtggtgaacttcattgtgcccttgacagtgatgttttactgttactaccacgtcagtcggtccctgagactctacgccgctagtgactgcactgcacacctccacagagactgggcagaccaggcagatgtaacaaagatgtctgtgataatgatactgatgtttctgctggcatggtccccttattccatcgtgtgcttgtgggcttgttttggaaaccccaaaaagattcctccttcaatggctatcatagctccactgtttgcaaaatcctctacgttctacaacccctgtatttacgtggctgcgcataagaagtttcggaaggccatgttggccatgtttaaatgccaacctcacctagcagtgcctgagccaagtactctaccaatggatatgcctcagagctcattggctcctgtgaggatctga

SEQ ID NO: 60 - DNA, 1080 bp, Gallus gallus
  source 1..1080: mol_type = genomic DNA
atggatgtattcagagcacttggaaatgagtcgctgttgtcgaactcctctggtcctgctcgatgggatcccttccaccatcccttggactccatccagccctggcacttcaggcttgtggcagcagtaatgttcgtggtgacctccctgtctcttgcggagaacctggctgtgatcctggtaacttttaagttcaagcagctgagacaacctgtcaattatgttatagtgaatttatctgtggctgatttcctggtctctttgactggtggcaccatcagctttttagccaacctaaaaggctatttctatatggggcactgggcttgtgtactggaaggatttgctgtcacgttttttggcattgtggctctctggtctcttgctcttttggcttttgagcggtacattgtgatctgccgcccagtgggaaatatgcgcttgagagggaagcatgctgcccaaggtattgcttttgtgtggaccttttccttcatttggaccattccaccaaccatgggttggagcagctacaccaccagtaagattggaactacttgtgagcctaattggtattcaggagcttataatgatcgttcctacattattgcattcttcaccacctgttttatagtgcctttattggtaattctggtgtcgtatgggaaactgctgcagaagctaagaaaggtgtcaaatacacaaggcaggttgagaactgccaggaaacctgaaagacaagtgactagaatggtggttgttatgatcattgcttttctaatctgctggatgccatatgccgtcttttctatcctagccactgcatacccttccattgaactggatcctcacctggcagcaattccagctttcttttccaaaacagctactgtttataatccaattatttatgtttttatgaacaaacagttcaggatgtgtctgattcagatgttcaagtgtagtgccatagagactgcggagtccaacatgaacccaacttcagagagagcaacactcacccaagacaaaagagacagtcagttgtctgtcatggcagtacgaagcaccatttcttag

SEQ ID NO: 61 - DNA, 1188 bp, Gallus gallus
  source 1..1188: mol_type = genomic DNA
atgcactcggggaacggcacgggggcgacgagccgcccgcagctcgcggcggcggggcacgaggtgccgggcgagcgtccgctcttcagcgccggcacctacgagctgctggcgctgctcatcgccaccatcggcacgctgggcgtgtgcaacaacttgctggtgctggtgctctactacaagttcaagcggctccgcacgcccaccaacctgttcctcgtcaacatcagcctcagcgacctgctggtgtccgtctgcggcgtcagcctcaccttcatgtcctgcctgcggagccgctgggtgtgggacgccgccggctgcgtctgggacggcttcagcaacagcctcttcgggatcgtttcaattatgactctcactgttcttgcctatgaacgctacattcgagtagtccatgcaaaagtgattgacttctcttggtcttggcgggctatcacatacatttggctttattcgttagcctggacaggagcacctcttttgggctggaacagatacacactggaaattcatggattaggttgctcaatggactggaagtcaaaagatcccaatgatacctcctttgtgctacttttcttccttggctgtctggtagcacctgttgtgatcatggcctattgctacggccatatcttatacgcagtaagaatgcttcgatgtgtggaagattttcagacttctcaagtgattaaacttctaaaatatgaaaagaaagtggctaaaatgtgtttcttaatgatctctaccttccttatttgttggatgccttatgcagtcgtctccctcctagtaacatatggctatagcaaccttgtaactcccacagtagctataatcccatctttctttgccaaatcaagtactgcttataatccagtcatctacatcttcatgagtagaaagtttcgacaatgccttttgcaactcctgtgctttcgcctgatgagattccagaggatcatgaaagagccctcaggagcagggaatgtcaaaccgatacgtccgatagtaatgtctcagaaagtaggggacaggccaaagaagaaagtgacattcagctcttcctccatcatttttattatcgccagtgatgacactcagcaaatagatgacaacagcaaacacaatgggacaaaagtaaatgtcatccaagtaaaaccactatag

SEQ ID NO: 62 - DNA, 1122 bp, Gallus gallus
  source 1..1122: mol_type = genomic DNA
atgaaccacacttggacatataacctgagctttggtgcacctacagatcctgttgagccaagagctggactgtcacgaaatgggcacacagtagtggctgtttttcttggatttatcttgttttttggtttcctgaataacttgattgtcctcatcctcttctgcaagtttaaaaccctccgtaaccctgtcaacatgcttctcctgaacatcagtatcagtgacatgttagtgtgcatctcaggcactaccctgagttttgcatctaacatccatggcaagtggattggaggggagcatggttgtaggtggtatggctttgtcaattcctgctttggcatcgtgtccctgatctccctggctgtcctgtcctacgaacgctacagcacccttaccctgtgtaacaagcgcagcgatgactatcggaaagcgctgctggcagttggcggttcttgggtttattccttgctctggactgtgccacctctgcttggatggagcagttatgggatagaaggtgcaggcaccagctgttcagtgcgctggtcctctgagacagctgagtccacgtcctatatcatctgtctcttcatattctgcttggtcatccctgtaatggtcatgatgtactgctatggtcggctcctttatgctgtcaaacaggttggaaaaatccacaagaacactgctcgcaaaagagaataccacgtactgttcatggtgatcactacagttatctgttatcttgtatgttggattccctatggagttatagcactacttgcaacatttggtaagccaggtgtggtgactccagttgcaagcatcataccttccatcttagcaaaaagcagcactgtttgcaatcccattatctacatacttatgaataagcagttttacaaatgctttcgccagcttttccactgtcaacctccttcctcaactgatggagagcccacctgccactccaaggtaaccgttatccagctgaatcagaaaacagatggtggaaagttgtgcaataataaaccacgtccagaaacagacaataaagtcacttctcttctgcacccagaaccaggcctggagccagctgcaaaaactgtaccaccaatgtaa

SEQ ID NO: 63 - DNA, 1632 bp, Gallus gallus
  source 1..1632: mol_type = genomic DNA
atggatttgaacatgggcacccagccacattctgtgaccaagtcagagatcccagaccatgttctttacacggtggggacgtgtgttcttgttattggctccattggcatcataggaaacctcctagttctctatgcattttacagcaacaagaagctgaggacaccccagaacttctttataatgaatttggctgtgagtgacttcctgatgtcagcttctcaggcccccatatgctttatcaacagcttgcacagagagtggatccttggagatataggttgtgacttgtatgctttctgcggggcgctctttggaataacctcgatgatgactctgttagctatttctgttgaccgctatttggtgatcaccaagcccctgcgctccatccagtggacctccaagaagcgcaccatacagattattgctgctgtgtggctgtactcgctggggtggagcgtagccccactccttgggtggagttcctacgtgcctgagggcttgatgatatcctgtacatgggactatgtaacctactcccctgcaaatagaagttacaccatgattttatgctgctgcgtattttttattcccctgataataatactccattgctatttatttatgttcttggccataagaagtactggcagagatgtccaaaagcttgggtcctgcagccgcaaatccttcctctctcagtccatgaagaatgaatggaaactggcaaaaattgcgtttgtggtcatcattgtgtatgtcttgtcctggtctccatatgcttgtgtcaccttgattgcctgggcaggccgaggaaacactctaacgccgtattccaaatctgtgccagctgttattgctaaagcctctgcaatctacaaccccatcatatatgcaataattcacccgagatacagaaaaaccatccacaatgctgtgccctgcttaaggttcctaatacgaatatcaaagaatgatctcctgagaggctccataaatgaatcatcattcaggacctctctctccagccaccagtctcttgctggaaggaccaagaacacttgtgtttcatcagtttccactggagaagctaactggagtgatgtagagcttgacactgtagaaccagctcatgagaaactgcagcctcgccgaagtcattccttctcatcaagtctgagacagaagagagacctgcttccagacagctatagctgcagtgaagaaactgaagaaaaggtttcgctgtcatccagctacctggagaaggtgctggggcgatcagccttccccagctcccctgtagcacttgtgaccagctccctccgagcagcctctcttcccgttggtttgaacagcagcagtgccagcagaggagcaggctcagatatctcacagatgaaaactgaagaaagtcataataatggaggcctggactccattgttagtaatacagtccctcaaatcattatcattcctacctcagagacaaacctatttcaagaggaacctgaagaggaagagactgaattattccacttccatgacaaaaagaacaatctgctggatttggaagggcttagctcatctacagagttcctcgaagctgttgagaaatttctatcataa

SEQ ID NO: 64 - DNA, 1587 bp, Gallus gallus
  source 1..1587: mol_type = genomic DNA
atggacctgcctcctagagccccaacaaagatgacagtgaaagatgttcgtggtgcttttcctacggtggacgtcccagaccatgcccattatacaattggaacagtcattcttatcgtggggatcacaggaactctgggtaatttcctggtcatctatgctttctgcaggagtaggacccttcagaaaccagccaatatattcatcatcaatctagctgttagtgacttccttatgtccattacacagtctccagtatttttcaccaacagtctccataaacgttggatttttggtgagaaaggctgtgagctgtatgccttctgcggagctctttttggcattacatccatgatcactttgatggtgattgccttggacagatactttgtcatcacaaaacctctggcttctgttcgagtgatgtcaaagaagaaggcccttataatcctggtaggcgtctggctgtactctttggcttggagcctcccacccttctttggatggagtgcctatgttcctgaaggcctgctgacttcctgttcctgggattacatgactttcacaccatcagtccgtgcctacacaatgctgcttttctgctttgtcttcttcattcctttgattgctatcatatacagctatgtctttatatttgaggctatcaagaaggccaacaagtctgtacagacatttggttgcaaacatggaaacagagagctccagaaacagtatcataggatgaggaatgagtggaagttggccaagattgcactgatcgtcatcttgctttatgtcatttcctggtcaccatactctgttgttgccctggtagcttttgctgggtattctcatgttctaacacctttcatgaattcagtaccagctgtgattgccaaagcttctgccatccataaccccattatttatgccatcactcaccctaaatatagaacagccattgcaacatatgtaccctgccttggattcctgctgagagtttctcctaaagagtcacgatcctttagcagttatccctcctccagacgaaccaccataaccagccagtcttctgagacaagtgggctgcagaaaggaaaaaggcgactatcttccatctctgatagtgaatcgggctgtaccgatacagaaactgatatcaccagtatgatctccagacctgctagcagccaggtttcctatgaaatgggggaagatacaacccaaactagtgacctaggaggcaaacctaaagtgaaaagccatgattctgggattttcaggaagacagttgtagatgcagatgaaatacccatggtggaaatcaatgacacagagcattctgctacatctacttgcaaaacatctgaaaaatgcaatgtggaggaaattcagagaagtgagagcctgagtggtattggactaagagaaggagagtctcgccatagaacatccgcatctcagatacccagcattataataacatacagcaacgtacaaggagtagagctgccttcaggatacagtgctggcttcctgcacccaaagaacaaaagccacaaacagaacaagagctccaacagctga

SEQ ID NO: 65 - DNA, 1074 bp, Gallus gallus
  source 1..1074: mol_type = genomic DNA
atgagtgggatggcatcggactgcaactcctcctctcaggaagaatacctcccacactacgtgcagcaggaagacccctttgcatcaaagctgtctagagaagctgacatcatagcggggttttatttgacagtaattgggattctttcaactctgggaaacgggtatgttatctttatgtcctcaaagcggaaaaagaagttaagacccgctgagataatgactgttaatttagcggtgtgtgatctgggcatctcagttgtaggaaaacccttcagtatcatttccttcttttctcaccgctggatctttggatggatgggctgccgctggtacggatgggctggcttcttctttggctgtgggagccttattaccatgacagccgtcagcctggatagatacttaaaaatctgtcacttggcttatggtacctggcttaagagacaccatgcctttatctgcctggcactaatctgggcctatgcgacgttctgggctacagtgccttttgctggtgtggggagctacgctcctgagccgtttgggacctcgtgcaccctggactggtggctggcgcaggcttcagtggctgggcaggcttttgttctcagcattcttttcttttgcctcctgtttccaactgcagtgattgtgttctcctatgttaaaattattttaaaagtcaagtcgtccaccaaagaagttgctcactatgacaccaggatccagaacagccacatacttgaaatgaagctgaccaaggtggcaatgctgatctgtgccggattcctcattgcttggatcccctacgccgtggtctctgtgtggtcagcctttggacagccggattccgttcccattcaattttcggtggtaccaactctgcttgccaagtcggctgccatgtacaacccaattatttaccaggtcattgattgcaaatttgcctgctgccggtcaggtgggccgaagacactgcagaagaagagctctttgaaggaatcgaggatgtacaccttatcttcacacagagattcagcggcactgagcggaacccaactggaagtctga

SEQ ID NO: 66 - DNA, 1047 bp, Gallus gallus
  source 1..1047: mol_type = genomic DNA
atggaggagcagtacatttccaaactgcacccggtagtggactacggagctggggtctttcttctgatcatagccatcctgacaatccttggaaattccgctgtccttgctacagcagtgaaacgctcttccctcctgaagtcaccagagctgcttacagtcaacctggcagtagcagatattgggatggcaatcagcatgtacccgctggcaattgcatctgcctggaaccacgcttggctgggaggagatgcgtcctgcatatattacgccctgatgggtttcctttttggtgtctgcagcatgatgacgctgtgtgccatggctgtgattcgattccttgttaccaattcatccaaatctaacagtaacaaaatctctaagaatactgttcacatcctgattactttcatctggctctactccttgctctgggccattctacccttggtaggctggggctactatggccccgagccatttggcatctcttgtacgatagcctggagcaagttccacagctcctccaatggcttttcattcatcctgagcatgttcctcctgtgcacagtcctgcctgctctgaccatcgtcgcctgttacttgggaattgcctggaaggttcataaagcataccaagagatccagaatatcaacaggattcctcacgcagctaaactggagaagaagctgacattgatggctgtgctcatctcagttgggttcctgagcgcatggacgccgtatgcagcagccagcttctggtccatatttaactccagcgattccctgcagcccattgtcacgctgctgccgtgtctgtttgccaaatcttcaaccgcgtataacccttttatttactacatcttcagcaaaactttccgtcatgaaatcaaacagctgcagtgctgctggggctggcgagttcatttcttcagcgctgataactctgcagaaaattccgtctcgatgatgtggagtgggagagataacatacgtctctcccccactgcaaaggtggagagccaaggagctgcaaggcactga

SEQ ID NO: 67 - DNA, 1005 bp, Gallus gallus
  source 1..1005: mol_type = genomic DNA
atgcattggaatgattcagccaactcctccgaaagtgatgctgaagctcattctgtctttacacagactgagcacaacatagtcgcagcttacttaataacagcaggagtgataagcattttcagcaatattgttgtgttaggcatctttgtgaagtacaaagagtttcggacagcaaccaatgcaattattatcaacctggctttcactgacattggtgttagtggcattggctaccccatgtctgctgcttcagacctgcatggaagctggaagtttggatatactggatgccagatctatgctgccttaaatatattttttgggatggcgagtattggtttgctcactgttgttgcagttgaccgttacctgacaatctgcaggcctgacataggaagaagaatgactacccgtaactatgccgctctaatcctggctgcgtggatcaacgcagtcttttgggcgtccatgcctactgtaggctgggctggctatgcttcagatccgactggagcaacttgcacagccaattggaggaaaaatgatgtgccctttgtttcctacacaatgagtgtaattgctgttaattttgttgtacccttaacagtcatgttttactgttattacaatgtttcccggacaatgaaacaatacaccagcagtaactgcctggagagcatcaacatggattggtctgaccaagtagatgtaacaaagatgtctgttgtgatgattgtcatgttcctggtggcatggtctccctattccattgtgtgtctatggtcttcctttggagacccgaagaaaatttctcctgcaatggccatcatagctcctttatttgcaaaatcctccacgttctataatccctgcatttacgtcattgcaaacaaaaagtttcggagagcaatcctggcaatggtgcgatgtcagacaagacaagaaataactataagcaatgccttgcccatgactgtttctctgagtgcattgacgtcataa

SEQ ID NO: 68 - DNA, 888 bp, Gallus gallus
  source 1..888: mol_type = genomic DNA
atggtcacttcacatcctctccctgaaggcttcactgaaatagaggtgtttgccatcggcactgccctactggtagaagccctgcttggtttctgtctgaatggcttgacgattatttcattccgaaaaatcaaagagctccgaacacccagcaacctgctggttctcagcatcgcactggctgactgcgggatatgcatcaatgcattcatcgctgccttttccagcttcctcaggtactggccctatggctccgagggctgtcagattcatggattccagggcttcttgacagcactagccagcatcagctccagcgcagcagttgcctgggaccggtatcatcactactgtacaaggagcaagctgcagtggagcacagccatctccatgatggtgttcgcgtggctgttcgctgccttctgggccacaatgcccttgctgggctggggggagtatgactatgagcccctccgaacctgctgcaccctggactacagcaaaggggacagaaactatatcacattcctttttgctctgtccattttcaatttcatgatcccgggcttcatcatgatgacggcctatcagtccatacatcagaagttcaagaaaagtgggcactataagtttaacactggcttaccgttgaagacgctggtcatttgctggggtccctactgccttctgagtttctatgcagcaattgaaaacgtgatgttcatttcaccaaaataccgaatgattcctgccattattgccaagacagtgccaaccgtggacagctttgtgtatgccctgggcaatgagaactacagaggaggaatatggcagttcctcacaggacagaagattgagaaagcagaggttgatagcaaaactaagtaa